European Patent Specification EP 3 783 022 B1, published March 4, 2026. Title: ANTI-VEGF-A ANTIBODIES AND USES THEREOF. Applicant: MEDIMMUNE LIMITED. Application PCT/EP2017/071106. The sequence listing filed with the application follows.

SEQUENCE LISTING (118 sequences)

SEQ ID NO: 1 - protein, 452 aa, Artificial Sequence
  source: /note="Description of Artificial Sequence: Synthetic polypeptide"
EVQLLESGGGLVQPGGSLRLSCAASGFTFSWYEMYWVRQAPGKGLEWVSSISPSGGWTMYADSVKGRFTISRDNSKNTLYLQMNSLRAEDTAVYYCATPLYSSDGLSAGDIWGQGTMVTVSSASTKGPSVFPLAPSSKSTSGGTAALGCLVKDYFPEPVTVSWNSGALTSGVHTFPAVLQSSGLYSLSSVVTVPSSSLGTQTYICNVNHKPSNTKVDKRVEPKSCDKTHTCPPCPAPELLGGPSVFLFPPKPKDTLMISRTPEVTCVVVDVSHEDPEVKFNWYVDGVEVHNAKTKPREEQYNSTYRVVSVLTVLHQDWLNGKEYKCKVSNKALPAPIEKTISKAKGQPREPQVYTLPPSREEMTKNQVSLTCLVKGFYPSDIAVEWESNGQPENNYKTTPPVLDSDGSFFLYSKLTVDKSRWQQGNVFSCSVMHEALHNHYTQKSLSLSPGK

SEQ ID NO: 2 - DNA, 1356 bp, Artificial Sequence
  source: /note="Description of Artificial Sequence: Synthetic polynucleotide"
gaggtgcagctgctggagagcggcggcggcctggtgcagcccggcggcagcctgaggctgagctgcgccgccagcggcttcaccttcagctggtacgagatgtactgggtgaggcaggcccccggcaagggcctggagtgggtgagcagcatcagccccagcggcggctggaccatgtacgccgacagcgtgaagggcaggttcaccatcagcagggacaacagcaagaacaccctgtacctgcagatgaacagcctgagggccgaggacaccgccgtgtactactgcgccacccccctgtacagcagcgacggcctgagcgccggcgacatctggggccagggcaccatggtgaccgtgagcagcgccagcaccaagggccccagcgtgttccccctggcccccagcagcaagagcaccagcggcggcaccgccgccctgggctgcctggtgaaggactacttccccgagcccgtgaccgtgagctggaacagcggcgccctgaccagcggcgtgcacaccttccccgccgtgctgcagagcagcggcctgtacagcctgagcagcgtggtgaccgtgcccagcagcagcctgggcacccagacctacatctgcaacgtgaaccacaagcccagcaacaccaaggtggacaagagggtggagcccaagagctgcgacaagacccacacctgccccccctgccccgcccccgagctgctgggcggccccagcgtgttcctgttcccccccaagcccaaggacaccctgatgatcagcaggacccccgaggtgacctgcgtggtggtggacgtgagccacgaggaccccgaggtgaagttcaactggtacgtggacggcgtggaggtgcacaacgccaagaccaagcccagggaggagcagtacaacagcacctacagggtggtgagcgtgctgaccgtgctgcaccaggactggctgaacggcaaggagtacaagtgcaaggtgagcaacaaggccctgcccgcccccatcgagaagaccatcagcaaggccaagggccagcccagggagccccaggtgtacaccctgccccccagcagggaggagatgaccaagaaccaggtgagcctgacctgcctggtgaagggcttctaccccagcgacatcgccgtggagtgggagagcaacggccagcccgagaacaactacaagaccaccccccccgtgctggacagcgacggcagcttcttcctgtacagcaagctgaccgtggacaagagcaggtggcagcagggcaacgtgttcagctgcagcgtgatgcacgaggccctgcacaaccactacacccagaagagcctgagcctgagccccggcaag

SEQ ID NO: 3 - protein, 122 aa, Artificial Sequence
  source: /note="Description of Artificial Sequence: Synthetic polypeptide"
EVQLLESGGGLVQPGGSLRLSCAASGFTFSWYEMYWVRQAPGKGLEWVSSISPSGGWTMYADSVKGRFTISRDNSKNTLYLQMNSLRAEDTAVYYCATPLYSSDGLSAGDIWGQGTMVTVSS

SEQ ID NO: 4 - DNA, 366 bp, Artificial Sequence
  source: /note="Description of Artificial Sequence: Synthetic polynucleotide"
gaggtgcagctgctggagagcggcggcggcctggtgcagcccggcggcagcctgaggctgagctgcgccgccagcggcttcaccttcagctggtacgagatgtactgggtgaggcaggcccccggcaagggcctggagtgggtgagcagcatcagccccagcggcggctggaccatgtacgccgacagcgtgaagggcaggttcaccatcagcagggacaacagcaagaacaccctgtacctgcagatgaacagcctgagggccgaggacaccgccgtgtactactgcgccacccccctgtacagcagcgacggcctgagcgccggcgacatctggggccagggcaccatggtgaccgtgagcagc

SEQ ID NO: 5 - protein, 214 aa, Artificial Sequence
  source: /note="Description of Artificial Sequence: Synthetic polypeptide"
DIQMTQSPATLSLSPGERATLSCRASQSVSSSYLAWYQQKPGQAPRLLIYGASSRATGIPDRFSGSGSGTDFTLTISRLEPEDFATYYCQQSYSTPSFGQGTRLEITRTVAAPSVFIFPPSDEQLKSGTASVVCLLNNFYPREAKVQWKVDNALQSGNSQESVTEQDSKDSTYSLSSTLTLSKADYEKHKVYACEVTHQGLSSPVTKSFNRGEC

SEQ ID NO: 6 - DNA, 642 bp, Artificial Sequence
  source: /note="Description of Artificial Sequence: Synthetic polynucleotide"
gacatccagatgacccagagccccgccaccctgagcctgagccccggcgagagggccaccctgagctgcagggccagccagagcgtgagcagcagctacctggcctggtaccagcagaagcccggccaggcccccaggctgctgatctacggcgccagcagcagggccaccggcatccccgacaggttcagcggcagcggcagcggcaccgacttcaccctgaccatcagcaggctggagcccgaggacttcgccacctactactgccagcagagctacagcacccccagcttcggccagggcaccaggctggagatcaccaggaccgtggccgcccccagcgtgttcatcttcccccccagcgacgagcagctgaagagcggcaccgccagcgtggtgtgcctgctgaacaacttctaccccagggaggccaaggtgcagtggaaggtggacaacgccctgcagagcggcaacagccaggagagcgtgaccgagcaggacagcaaggacagcacctacagcctgagcagcaccctgaccctgagcaaggccgactacgagaagcacaaggtgtacgcctgcgaggtgacccaccagggcctgagcagccccgtgaccaagagcttcaacaggggcgagtgc

SEQ ID NO: 7 - protein, 107 aa, Artificial Sequence
  source: /note="Description of Artificial Sequence: Synthetic polypeptide"
DIQMTQSPATLSLSPGERATLSCRASQSVSSSYLAWYQQKPGQAPRLLIYGASSRATGIPDRFSGSGSGTDFTLTISRLEPEDFATYYCQQSYSTPSFGQGTRLEIT

SEQ ID NO: 8 - DNA, 321 bp, Artificial Sequence
  source: /note="Description of Artificial Sequence: Synthetic polynucleotide"
gacatccagatgacccagagccccgccaccctgagcctgagccccggcgagagggccaccctgagctgcagggccagccagagcgtgagcagcagctacctggcctggtaccagcagaagcccggccaggcccccaggctgctgatctacggcgccagcagcagggccaccggcatccccgacaggttcagcggcagcggcagcggcaccgacttcaccctgaccatcagcaggctggagcccgaggacttcgccacctactactgccagcagagctacagcacccccagcttcggccagggcaccaggctggagatcacc

SEQ ID NO: 9 - protein, 5 aa, Artificial Sequence
  source: /note="Description of Artificial Sequence: Synthetic peptide"
WYEMY

SEQ ID NO: 10 - protein, 17 aa, Artificial Sequence
  source: /note="Description of Artificial Sequence: Synthetic peptide"
SISPSGGWTMYADSVKG

SEQ ID NO: 11 - protein, 13 aa, Artificial Sequence
  source: /note="Description of Artificial Sequence: Synthetic peptide"
PLYSSDGLSAGDI

SEQ ID NO: 12 - protein, 12 aa, Artificial Sequence
  source: /note="Description of Artificial Sequence: Synthetic peptide"
RASQSVSSSYLA

SEQ ID NO: 13 - protein, 7 aa, Artificial Sequence
  source: /note="Description of Artificial Sequence: Synthetic peptide"
GASSRAT

SEQ ID NO: 14 - protein, 8 aa, Artificial Sequence
  source: /note="Description of Artificial Sequence: Synthetic peptide"
QQSYSTPS

SEQ ID NO: 15 - protein, 452 aa, Artificial Sequence; identical to SEQ ID NO: 1
  source: /note="Description of Artificial Sequence: Synthetic polypeptide"

SEQ ID NO: 16 - DNA, 1356 bp, Artificial Sequence; identical to SEQ ID NO: 2
  source: /note="Description of Artificial Sequence: Synthetic polynucleotide"

SEQ ID NO: 17 - protein, 122 aa, Artificial Sequence; identical to SEQ ID NO: 3
  source: /note="Description of Artificial Sequence: Synthetic polypeptide"

SEQ ID NO: 18 - DNA, 366 bp, Artificial Sequence; identical to SEQ ID NO: 4
  source: /note="Description of Artificial Sequence: Synthetic polynucleotide"

SEQ ID NO: 19 - protein, 214 aa, Artificial Sequence
  source: /note="Description of Artificial Sequence: Synthetic polypeptide"
EIVLTQSPATLSLSPGERATLSCRASQSVSSSYLAWYQQKPGQAPRLLIYGASSRATGIPDRFSGSGSGTDFTLTISRLEPEDFAVYYCQQSYSTPSFGQGTRLEITRTVAAPSVFIFPPSDEQLKSGTASVVCLLNNFYPREAKVQWKVDNALQSGNSQESVTEQDSKDSTYSLSSTLTLSKADYEKHKVYACEVTHQGLSSPVTKSFNRGEC

SEQ ID NO: 20 - DNA, 642 bp, Artificial Sequence
  source: /note="Description of Artificial Sequence: Synthetic polynucleotide"
gagatcgtgctgacccagagccccgccaccctgagcctgagccccggcgagagggccaccctgagctgcagggccagccagagcgtgagcagcagctacctggcctggtaccagcagaagcccggccaggcccccaggctgctgatctacggcgccagcagcagggccaccggcatccccgacaggttcagcggcagcggcagcggcaccgacttcaccctgaccatcagcaggctggagcccgaggacttcgccgtgtactactgccagcagagctacagcacccccagcttcggccagggcaccaggctggagatcaccaggaccgtggccgcccccagcgtgttcatcttcccccccagcgacgagcagctgaagagcggcaccgccagcgtggtgtgcctgctgaacaacttctaccccagggaggccaaggtgcagtggaaggtggacaacgccctgcagagcggcaacagccaggagagcgtgaccgagcaggacagcaaggacagcacctacagcctgagcagcaccctgaccctgagcaaggccgactacgagaagcacaaggtgtacgcctgcgaggtgacccaccagggcctgagcagccccgtgaccaagagcttcaacaggggcgagtgc

SEQ ID NO: 21 - protein, 107 aa, Artificial Sequence
  source: /note="Description of Artificial Sequence: Synthetic polypeptide"
EIVLTQSPATLSLSPGERATLSCRASQSVSSSYLAWYQQKPGQAPRLLIYGASSRATGIPDRFSGSGSGTDFTLTISRLEPEDFAVYYCQQSYSTPSFGQGTRLEIT

SEQ ID NO: 22 - DNA, 321 bp, Artificial Sequence
  source: /note="Description of Artificial Sequence: Synthetic polynucleotide"
gagatcgtgctgacccagagccccgccaccctgagcctgagccccggcgagagggccaccctgagctgcagggccagccagagcgtgagcagcagctacctggcctggtaccagcagaagcccggccaggcccccaggctgctgatctacggcgccagcagcagggccaccggcatccccgacaggttcagcggcagcggcagcggcaccgacttcaccctgaccatcagcaggctggagcccgaggacttcgccgtgtactactgccagcagagctacagcacccccagcttcggccagggcaccaggctggagatcacc

SEQ ID NO: 23 - protein, 5 aa, Artificial Sequence
  source: /note="Description of Artificial Sequence: Synthetic peptide"
WYEMY

SEQ ID NO: 24 - protein, 17 aa, Artificial Sequence
  source: /note="Description of Artificial Sequence: Synthetic peptide"
SISPSGGWTMYADSVKG

SEQ ID NO: 25 - protein, 13 aa, Artificial Sequence
  source: /note="Description of Artificial Sequence: Synthetic peptide"
PLYSSDGLSAGDI

SEQ ID NO: 26 - protein, 12 aa, Artificial Sequence
  source: /note="Description of Artificial Sequence: Synthetic peptide"
RASQSVSSSYLA

SEQ ID NO: 27 - protein, 7 aa, Artificial Sequence
  source: /note="Description of Artificial Sequence: Synthetic peptide"
GASSRAT

SEQ ID NO: 28 - protein, 8 aa, Artificial Sequence
  source: /note="Description of Artificial Sequence: Synthetic peptide"
QQSYSTPS

SEQ ID NO: 29 - protein, 452 aa, Artificial Sequence; identical to SEQ ID NO: 1
  source: /note="Description of Artificial Sequence: Synthetic polypeptide"

SEQ ID NO: 30 - DNA, 1356 bp, Artificial Sequence; identical to SEQ ID NO: 2
  source: /note="Description of Artificial Sequence: Synthetic polynucleotide"

SEQ ID NO: 31 - protein, 122 aa, Artificial Sequence; identical to SEQ ID NO: 3
  source: /note="Description of Artificial Sequence: Synthetic polypeptide"

SEQ ID NO: 32 - DNA, 366 bp, Artificial Sequence; identical to SEQ ID NO: 4
  source: /note="Description of Artificial Sequence: Synthetic polynucleotide"

SEQ ID NO: 33 - protein, 214 aa, Artificial Sequence
  source: /note="Description of Artificial Sequence: Synthetic polypeptide"
EIVLTQSPATLSLSPGERATLSCRASQSVHSSYLAWYQQKPGQAPRLLIYGASSRATGIPDRFSGSGSGTDFTLTISRLEPEDFAVYYCQQSYSTPSFGQGTRLEITRTVAAPSVFIFPPSDEQLKSGTASVVCLLNNFYPREAKVQWKVDNALQSGNSQESVTEQDSKDSTYSLSSTLTLSKADYEKHKVYACEVTHQGLSSPVTKSFNRGEC

SEQ ID NO: 34 - DNA, 642 bp, Artificial Sequence
  source: /note="Description of Artificial Sequence: Synthetic polynucleotide"
gagatcgtgctgacccagagccccgccaccctgagcctgagccccggcgagagggccaccctgagctgcagggccagccagagcgtgcacagcagctacctggcctggtaccagcagaagcccggccaggcccccaggctgctgatctacggcgccagcagcagggccaccggcatccccgacaggttcagcggcagcggcagcggcaccgacttcaccctgaccatcagcaggctggagcccgaggacttcgccgtgtactactgccagcagagctacagcacccccagcttcggccagggcaccaggctggagatcaccaggaccgtggccgcccccagcgtgttcatcttcccccccagcgacgagcagctgaagagcggcaccgccagcgtggtgtgcctgctgaacaacttctaccccagggaggccaaggtgcagtggaaggtggacaacgccctgcagagcggcaacagccaggagagcgtgaccgagcaggacagcaaggacagcacctacagcctgagcagcaccctgaccctgagcaaggccgactacgagaagcacaaggtgtacgcctgcgaggtgacccaccagggcctgagcagccccgtgaccaagagcttcaacaggggcgagtgc

SEQ ID NO: 35 - protein, 107 aa, Artificial Sequence
  source: /note="Description of Artificial Sequence: Synthetic polypeptide"
EIVLTQSPATLSLSPGERATLSCRASQSVHSSYLAWYQQKPGQAPRLLIYGASSRATGIPDRFSGSGSGTDFTLTISRLEPEDFAVYYCQQSYSTPSFGQGTRLEIT

SEQ ID NO: 36 - DNA, 321 bp, Artificial Sequence
  source: /note="Description of Artificial Sequence: Synthetic polynucleotide"
gagatcgtgctgacccagagccccgccaccctgagcctgagccccggcgagagggccaccctgagctgcagggccagccagagcgtgcacagcagctacctggcctggtaccagcagaagcccggccaggcccccaggctgctgatctacggcgccagcagcagggccaccggcatccccgacaggttcagcggcagcggcagcggcaccgacttcaccctgaccatcagcaggctggagcccgaggacttcgccgtgtactactgccagcagagctacagcacccccagcttcggccagggcaccaggctggagatcacc

SEQ ID NO: 37 - protein, 5 aa, Artificial Sequence
  source: /note="Description of Artificial Sequence: Synthetic peptide"
WYEMY

SEQ ID NO: 38 - protein, 17 aa, Artificial Sequence
  source: /note="Description of Artificial Sequence: Synthetic peptide"
SISPSGGWTMYADSVKG

SEQ ID NO: 39 - protein, 13 aa, Artificial Sequence
  source: /note="Description of Artificial Sequence: Synthetic peptide"
PLYSSDGLSAGDI

SEQ ID NO: 40 - protein, 12 aa, Artificial Sequence
  source: /note="Description of Artificial Sequence: Synthetic peptide"
RASQSVHSSYLA

SEQ ID NO: 41 - protein, 7 aa, Artificial Sequence
  source: /note="Description of Artificial Sequence: Synthetic peptide"
GASSRAT

SEQ ID NO: 42 - protein, 8 aa, Artificial Sequence
  source: /note="Description of Artificial Sequence: Synthetic peptide"
QQSYSTPS

SEQ ID NO: 43 - protein, 452 aa, Artificial Sequence; identical to SEQ ID NO: 1
  source: /note="Description of Artificial Sequence: Synthetic polypeptide"

SEQ ID NO: 44 - DNA, 1356 bp, Artificial Sequence; identical to SEQ ID NO: 2
  source: /note="Description of Artificial Sequence: Synthetic polynucleotide"

SEQ ID NO: 45 - protein, 122 aa, Artificial Sequence; identical to SEQ ID NO: 3
  source: /note="Description of Artificial Sequence: Synthetic polypeptide"

SEQ ID NO: 46 - DNA, 366 bp, Artificial Sequence; identical to SEQ ID NO: 4
  source: /note="Description of Artificial Sequence: Synthetic polynucleotide"

SEQ ID NO: 47 - protein, 214 aa, Artificial Sequence
  source: /note="Description of Artificial Sequence: Synthetic polypeptide"
EIVLTQSPATLSLSPGERATLSCRASQSVSSSYLAWYQQKPGQAPRLLIYGASSRATGIPDRFSGSGSGTDFTLTISRLEPEDFAVYYCQQSYRTPSFGQGTRLEITRTVAAPSVFIFPPSDEQLKSGTASVVCLLNNFYPREAKVQWKVDNALQSGNSQESVTEQDSKDSTYSLSSTLTLSKADYEKHKVYACEVTHQGLSSPVTKSFNRGEC

SEQ ID NO: 48 - DNA, 642 bp, Artificial Sequence
  source: /note="Description of Artificial Sequence: Synthetic polynucleotide"
gagatcgtgctgacccagagccccgccaccctgagcctgagccccggcgagagggccaccctgagctgcagggccagccagagcgtgagcagcagctacctggcctggtaccagcagaagcccggccaggcccccaggctgctgatctacggcgccagcagcagggccaccggcatccccgacaggttcagcggcagcggcagcggcaccgacttcaccctgaccatcagcaggctggagcccgaggacttcgccgtgtactactgccagcagagctacaggacccccagcttcggccagggcaccaggctggagatcaccaggaccgtggccgcccccagcgtgttcatcttcccccccagcgacgagcagctgaagagcggcaccgccagcgtggtgtgcctgctgaacaacttctaccccagggaggccaaggtgcagtggaaggtggacaacgccctgcagagcggcaacagccaggagagcgtgaccgagcaggacagcaaggacagcacctacagcctgagcagcaccctgaccctgagcaaggccgactacgagaagcacaaggtgtacgcctgcgaggtgacccaccagggcctgagcagccccgtgaccaagagcttcaacaggggcgagtgc

SEQ ID NO: 49 - protein, 107 aa, Artificial Sequence
  source: /note="Description of Artificial Sequence: Synthetic polypeptide"
EIVLTQSPATLSLSPGERATLSCRASQSVSSSYLAWYQQKPGQAPRLLIYGASSRATGIPDRFSGSGSGTDFTLTISRLEPEDFAVYYCQQSYRTPSFGQGTRLEIT

SEQ ID NO: 50 - DNA, 321 bp, Artificial Sequence
  source: /note="Description of Artificial Sequence: Synthetic polynucleotide"
gagatcgtgctgacccagagccccgccaccctgagcctgagccccggcgagagggccaccctgagctgcagggccagccagagcgtgagcagcagctacctggcctggtaccagcagaagcccggccaggcccccaggctgctgatctacggcgccagcagcagggccaccggcatccccgacaggttcagcggcagcggcagcggcaccgacttcaccctgaccatcagcaggctggagcccgaggacttcgccgtgtactactgccagcagagctacaggacccccagcttcggccagggcaccaggctggagatcacc

SEQ ID NO: 51 - protein, 5 aa, Artificial Sequence
  source: /note="Description of Artificial Sequence: Synthetic peptide"
WYEMY

SEQ ID NO: 52 - protein, 17 aa, Artificial Sequence
  source: /note="Description of Artificial Sequence: Synthetic peptide"
SISPSGGWTMYADSVKG

SEQ ID NO: 53 - protein, 13 aa, Artificial Sequence
  source: /note="Description of Artificial Sequence: Synthetic peptide"
PLYSSDGLSAGDI

SEQ ID NO: 54 - protein, 12 aa, Artificial Sequence
  source: /note="Description of Artificial Sequence: Synthetic peptide"
RASQSVSSSYLA

SEQ ID NO: 55 - protein, 7 aa, Artificial Sequence
  source: /note="Description of Artificial Sequence: Synthetic peptide"
GASSRAT

SEQ ID NO: 56 - protein, 8 aa, Artificial Sequence
  source: /note="Description of Artificial Sequence: Synthetic peptide"
QQSYRTPS

SEQ ID NO: 57 - protein, 452 aa, Artificial Sequence; identical to SEQ ID NO: 1
  source: /note="Description of Artificial Sequence: Synthetic polypeptide"

SEQ ID NO: 58 - DNA, 1356 bp, Artificial Sequence; identical to SEQ ID NO: 2
  source: /note="Description of Artificial Sequence: Synthetic polynucleotide"

SEQ ID NO: 59 - protein, 122 aa, Artificial Sequence; identical to SEQ ID NO: 3
  source: /note="Description of Artificial Sequence: Synthetic polypeptide"

SEQ ID NO: 60 - DNA, 366 bp, Artificial Sequence; identical to SEQ ID NO: 4
  source: /note="Description of Artificial Sequence: Synthetic polynucleotide"

SEQ ID NO: 61 - protein, 214 aa, Artificial Sequence
  source: /note="Description of Artificial Sequence: Synthetic polypeptide"
EIVLTQSPATLSLSPGERATLSCRASQSVSSSYLAWYQQKPGQAPRLLIYGASSRATGIPDRFSGSGSGTDFTLTISRLEPEDFAVYYCQQDYSTPSFGQGTRLEITRTVAAPSVFIFPPSDEQLKSGTASVVCLLNNFYPREAKVQWKVDNALQSGNSQESVTEQDSKDSTYSLSSTLTLSKADYEKHKVYACEVTHQGLSSPVTKSFNRGEC

SEQ ID NO: 62 - DNA, 642 bp, Artificial Sequence
  source: /note="Description of Artificial Sequence: Synthetic polynucleotide"
gagatcgtgctgacccagagccccgccaccctgagcctgagccccggcgagagggccaccctgagctgcagggccagccagagcgtgagcagcagctacctggcctggtaccagcagaagcccggccaggcccccaggctgctgatctacggcgccagcagcagggccaccggcatccccgacaggttcagcggcagcggcagcggcaccgacttcaccctgaccatcagcaggctggagcccgaggacttcgccgtgtactactgccagcaggactacagcacccccagcttcggccagggcaccaggctggagatcaccaggaccgtggccgcccccagcgtgttcatcttcccccccagcgacgagcagctgaagagcggcaccgccagcgtggtgtgcctgctgaacaacttctaccccagggaggccaaggtgcagtggaaggtggacaacgccctgcagagcggcaacagccaggagagcgtgaccgagcaggacagcaaggacagcacctacagcctgagcagcaccctgaccctgagcaaggccgactacgagaagcacaaggtgtacgcctgcgaggtgacccaccagggcctgagcagccccgtgaccaagagcttcaacaggggcgagtgc

SEQ ID NO: 63 - protein, 107 aa, Artificial Sequence
  source: /note="Description of Artificial Sequence: Synthetic polypeptide"
EIVLTQSPATLSLSPGERATLSCRASQSVSSSYLAWYQQKPGQAPRLLIYGASSRATGIPDRFSGSGSGTDFTLTISRLEPEDFAVYYCQQDYSTPSFGQGTRLEIT

SEQ ID NO: 64 - DNA, 321 bp, Artificial Sequence
  source: /note="Description of Artificial Sequence: Synthetic polynucleotide"
gagatcgtgctgacccagagccccgccaccctgagcctgagccccggcgagagggccaccctgagctgcagggccagccagagcgtgagcagcagctacctggcctggtaccagcagaagcccggccaggcccccaggctgctgatctacggcgccagcagcagggccaccggcatccccgacaggttcagcggcagcggcagcggcaccgacttcaccctgaccatcagcaggctggagcccgaggacttcgccgtgtactactgccagcaggactacagcacccccagcttcggccagggcaccaggctggagatcacc

SEQ ID NO: 65 - protein, 5 aa, Artificial Sequence
  source: /note="Description of Artificial Sequence: Synthetic peptide"
WYEMY

SEQ ID NO: 66 - protein, 17 aa, Artificial Sequence
  source: /note="Description of Artificial Sequence: Synthetic peptide"
SISPSGGWTMYADSVKG

SEQ ID NO: 67 - protein, 13 aa, Artificial Sequence
  source: /note="Description of Artificial Sequence: Synthetic peptide"
PLYSSDGLSAGDI

SEQ ID NO: 68 - protein, 12 aa, Artificial Sequence
  source: /note="Description of Artificial Sequence: Synthetic peptide"
RASQSVSSSYLA

SEQ ID NO: 69 - protein, 7 aa, Artificial Sequence
  source: /note="Description of Artificial Sequence: Synthetic peptide"
GASSRAT

SEQ ID NO: 70 - protein, 8 aa, Artificial Sequence
  source: /note="Description of Artificial Sequence: Synthetic peptide"
QQDYSTPS

SEQ ID NO: 71 - protein, 452 aa, Artificial Sequence; identical to SEQ ID NO: 1
  source: /note="Description of Artificial Sequence: Synthetic polypeptide"

SEQ ID NO: 72 - DNA, 1356 bp, Artificial Sequence; identical to SEQ ID NO: 2
  source: /note="Description of Artificial Sequence: Synthetic polynucleotide"

SEQ ID NO: 73 - protein, 122 aa, Artificial Sequence; identical to SEQ ID NO: 3
  source: /note="Description of Artificial Sequence: Synthetic polypeptide"

SEQ ID NO: 74 - DNA, 366 bp, Artificial Sequence; identical to SEQ ID NO: 4
  source: /note="Description of Artificial Sequence: Synthetic polynucleotide"

SEQ ID NO: 75 - protein, 214 aa, Artificial Sequence
  source: /note="Description of Artificial Sequence: Synthetic polypeptide"
EIVLTQSPATLSLSPGERATLSCRASQSVHSSYLAWYQQKPGQAPRLLIYGASSRATGIPDRFSGSGSGTDFTLTISRLEPEDFAVYYCQQSYRTPSFGQGTRLEITRTVAAPSVFIFPPSDEQLKSGTASVVCLLNNFYPREAKVQWKVDNALQSGNSQESVTEQDSKDSTYSLSSTLTLSKADYEKHKVYACEVTHQGLSSPVTKSFNRGEC

SEQ ID NO: 76 - DNA, 642 bp, Artificial Sequence
  source: /note="Description of Artificial Sequence: Synthetic polynucleotide"
gagatcgtgctgacccagagccccgccaccctgagcctgagccccggcgagagggccaccctgagctgcagggccagccagagcgtgcacagcagctacctggcctggtaccagcagaagcccggccaggcccccaggctgctgatctacggcgccagcagcagggccaccggcatccccgacaggttcagcggcagcggcagcggcaccgacttcaccctgaccatcagcaggctggagcccgaggacttcgccgtgtactactgccagcagagctacaggacccccagcttcggccagggcaccaggctggagatcaccaggaccgtggccgcccccagcgtgttcatcttcccccccagcgacgagcagctgaagagcggcaccgccagcgtggtgtgcctgctgaacaacttctaccccagggaggccaaggtgcagtggaaggtggacaacgccctgcagagcggcaacagccaggagagcgtgaccgagcaggacagcaaggacagcacctacagcctgagcagcaccctgaccctgagcaaggccgactacgagaagcacaaggtgtacgcctgcgaggtgacccaccagggcctgagcagccccgtgaccaagagcttcaacaggggcgagtgc

SEQ ID NO: 77 - protein, 107 aa, Artificial Sequence
  source: /note="Description of Artificial Sequence: Synthetic polypeptide"
EIVLTQSPATLSLSPGERATLSCRASQSVHSSYLAWYQQKPGQAPRLLIYGASSRATGIPDRFSGSGSGTDFTLTISRLEPEDFAVYYCQQSYRTPSFGQGTRLEIT

SEQ ID NO: 78 - DNA, 321 bp, Artificial Sequence
  source: /note="Description of Artificial Sequence: Synthetic polynucleotide"
gagatcgtgctgacccagagccccgccaccctgagcctgagccccggcgagagggccaccctgagctgcagggccagccagagcgtgcacagcagctacctggcctggtaccagcagaagcccggccaggcccccaggctgctgatctacggcgccagcagcagggccaccggcatccccgacaggttcagcggcagcggcagcggcaccgacttcaccctgaccatcagcaggctggagcccgaggacttcgccgtgtactactgccagcagagctacaggacccccagcttcggccagggcaccaggctggagatcacc

SEQ ID NO: 79 - protein, 5 aa, Artificial Sequence
  source: /note="Description of Artificial Sequence: Synthetic peptide"
WYEMY

SEQ ID NO: 80 - protein, 17 aa, Artificial Sequence
  source: /note="Description of Artificial Sequence: Synthetic peptide"
SISPSGGWTMYADSVKG

SEQ ID NO: 81 - protein, 13 aa, Artificial Sequence
  source: /note="Description of Artificial Sequence: Synthetic peptide"
PLYSSDGLSAGDI

SEQ ID NO: 82 - protein, 12 aa, Artificial Sequence
  source: /note="Description of Artificial Sequence: Synthetic peptide"
RASQSVHSSYLA

SEQ ID NO: 83 - protein, 7 aa, Artificial Sequence
  source: /note="Description of Artificial Sequence: Synthetic peptide"
GASSRAT

SEQ ID NO: 84 - protein, 8 aa, Artificial Sequence
  source: /note="Description of Artificial Sequence: Synthetic peptide"
QQSYRTPS

SEQ ID NO: 85 - protein, 452 aa, Artificial Sequence; identical to SEQ ID NO: 1
  source: /note="Description of Artificial Sequence: Synthetic polypeptide"

SEQ ID NO: 86 - DNA, 1356 bp, Artificial Sequence
  source: /note="Description of Artificial Sequence: Synthetic polynucleotide"
gaagttcaattgttagagtctggtggcggtcttgttcagcctggtggttctttacgtctttcttgcgctgcttccggattcactttctcttggtacgagatgtattgggttcgccaagctcctggtaaaggtttggagtgggtttcttctatctctccttctggtggctggactatgtatgctgactccgttaaaggtcgcttcactatctctagagacaactctaagaatactctctacttgcagatgaacagcttaagggctgaggacacggccgtgtattactgtgcgacccccttgtatagcagtgacgggctttcggcgggggatatctggggccaagggacaatggtcaccgtctcaagcgcgtcgaccaagggcccatccgtcttccccctggcaccctcctccaagagcacctctgggggcacagcggccctgggctgcctggtcaaggactacttccccgaaccggtgacggtgtcctggaactcaggcgctctgaccagcggcgtgcacaccttcccggctgtcctacagtcctcaggactctactccctcagcagcgtggtgaccgtgccctccagcagcttgggcacccagacctacatctgcaacgtgaatcacaagcccagcaacaccaaggtggacaagagagttgagcccaaatcttgtgacaaaactcacacatgcccaccgtgcccagcacctgaactcctggggggaccgtcagtcttcctcttccccccaaaacccaaggacaccctcatgatctcccggacccctgaggtcacatgcgtggtggtggacgtgagccacgaagaccctgaggtcaagttcaactggtacgtggacggcgtggaggtgcataatgccaagacaaagccgcgggaggagcagtacaacagcacgtaccgtgtggtcagcgtcctcaccgtcctgcaccaggactggctgaatggcaaggagtacaagtgcaaggtctccaacaaagccctcccagcccccatcgagaaaaccatctccaaagccaaagggcagccccgagaaccacaggtctacaccctgcccccatcccgggaggagatgaccaagaaccaggtcagcctgacctgcctggtcaaaggcttctatcccagcgacatcgccgtggagtgggagagcaatgggcagccggagaacaactacaagaccacgcctcccgtgctggactccgacggctccttcttcctctatagcaagctcaccgtggacaagagcaggtggcagcaggggaacgtcttctcatgctccgtgatgcatgaggctctgcacaaccactacacgcagaagagcctctccctgtctccgggtaaa

SEQ ID NO: 87 - protein, 122 aa, Artificial Sequence; identical to SEQ ID NO: 3
  source: /note="Description of Artificial Sequence: Synthetic polypeptide"

SEQ ID NO: 88 - DNA, 366 bp, Artificial Sequence
  source: /note="Description of Artificial Sequence: Synthetic polynucleotide"
gaagttcaattgttagagtctggtggcggtcttgttcagcctggtggttctttacgtctttcttgcgctgcttccggattcactttctcttggtacgagatgtattgggttcgccaagctcctggtaaaggtttggagtgggtttcttctatctctccttctggtggctggactatgtatgctgactccgttaaaggtcgcttcactatctctagagacaactctaagaatactctctacttgcagatgaacagcttaagggctgaggacacggccgtgtattactgtgcgacccccttgtatagcagtgacgggctttcggcgggggatatctggggccaagggacaatggtcaccgtctcaagc

SEQ ID NO: 89 - protein, 214 aa, Artificial Sequence
  source: /note="Description of Artificial Sequence: Synthetic polypeptide"
EIVLTQSPATLSLSPGERATLSCRASQSVHSSYLAWYQQKPGQAPRLLIYGASSRATGIPDRFSGSGSGTDFTLTISRLEPEDFAVYYCQQSYRTPSFGQGTRLEIKRTVAAPSVFIFPPSDEQLKSGTASVVCLLNNFYPREAKVQWKVDNALQSGNSQESVTEQDSKDSTYSLSSTLTLSKADYEKHKVYACEVTHQGLSSPVTKSFNRGEC

SEQ ID NO: 90 - DNA, 642 bp, Artificial Sequence
  source: /note="Description of Artificial Sequence: Synthetic polynucleotide"
gagatcgtgctgacccagtctccagccaccctctctttgtctccaggggaaagagccaccctctcctgcagggccagtcagagtgttcacagcagctacttagcctggtaccagcagaaacctggccaggctcccaggctcctcatctatggtgcatccagcagggccactggcatcccagacaggttcagtggcagtgggtctgggacagacttcactctcaccatcagcagactggagcctgaagattttgcagtttactactgtcaacagagttaccgcaccccttccttcggccaagggacacgactggagattaaacgtacggtggctgcaccatctgtcttcatcttcccgccatctgatgagcagttgaaatctggaactgcctctgttgtgtgcctgctgaataacttctatcccagagaggccaaagtacagtggaaggtggataacgccctccaatcgggtaactcccaggagagtgtcacagagcaggacagcaaggacagcacctacagcctcagcagcaccctgacgctgagcaaagcagactacgagaaacacaaagtctacgcctgcgaagtcacccatcagggcctgagctcgcccgtcacaaagagcttcaacaggggagagtgt

SEQ ID NO: 91 - protein, 107 aa, Artificial Sequence
  source: /note="Description of Artificial Sequence: Synthetic polypeptide"
EIVLTQSPATLSLSPGERATLSCRASQSVHSSYLAWYQQKPGQAPRLLIYGASSRATGIPDRFSGSGSGTDFTLTISRLEPEDFAVYYCQQSYRTPSFGQGTRLEIK

SEQ ID NO: 92 - DNA, 321 bp, Artificial Sequence
  source: /note="Description of Artificial Sequence: Synthetic polynucleotide"
gagatcgtgctgacccagtctccagccaccctctctttgtctccaggggaaagagccaccctctcctgcagggccagtcagagtgttcacagcagctacttagcctggtaccagcagaaacctggccaggctcccaggctcctcatctatggtgcatccagcagggccactggcatcccagacaggttcagtggcagtgggtctgggacagacttcactctcaccatcagcagactggagcctgaagattttgcagtttactactgtcaacagagttaccgcaccccttccttcggccaagggacacgactggagattaaa

SEQ ID NO: 93 - protein, 5 aa, Artificial Sequence
  source: /note="Description of Artificial Sequence: Synthetic peptide"
WYEMY

SEQ ID NO: 94 - protein, 17 aa, Artificial Sequence
  source: /note="Description of Artificial Sequence: Synthetic peptide"
SISPSGGWTMYADSVKG

SEQ ID NO: 95 - protein, 13 aa, Artificial Sequence
  source: /note="Description of Artificial Sequence: Synthetic peptide"
PLYSSDGLSAGDI

SEQ ID NO: 96 - protein, 12 aa, Artificial Sequence
  source: /note="Description of Artificial Sequence: Synthetic peptide"
RASQSVHSSYLA

SEQ ID NO: 97 - protein, 7 aa, Artificial Sequence
  source: /note="Description of Artificial Sequence: Synthetic peptide"
GASSRAT

SEQ ID NO: 98 - protein, 8 aa, Artificial Sequence
  source: /note="Description of Artificial Sequence: Synthetic peptide"
QQSYRTPS

SEQ ID NO: 99 - protein, 452 aa, Artificial Sequence; identical to SEQ ID NO: 1
  source: /note="Description of Artificial Sequence: Synthetic polypeptide"

SEQ ID NO: 100 - DNA, 1356 bp, Artificial Sequence; identical to SEQ ID NO: 2
  source: /note="Description of Artificial Sequence: Synthetic polynucleotide"

SEQ ID NO: 101 - protein, 122 aa, Artificial Sequence; identical to SEQ ID NO: 3
  source: /note="Description of Artificial Sequence: Synthetic polypeptide"

SEQ ID NO: 102 - DNA, 366 bp, Artificial Sequence; identical to SEQ ID NO: 4
  source: /note="Description of Artificial Sequence: Synthetic polynucleotide"

SEQ ID NO: 103 - protein, 214 aa, Artificial Sequence
  source: /note="Description of Artificial Sequence: Synthetic polypeptide"
EIVLTQSPATLSLSPGERATLSCRASQSVHSSYLAWYQQKPGQAPRLLIYGASSRATGIPDRFSGSGSGTDFTLTISRLEPEDFAVYYCQQDYRTPSFGQGTRLEITRTVAAPSVFIFPPSDEQLKSGTASVVCLLNNFYPREAKVQWKVDNALQSGNSQESVTEQDSKDSTYSLSSTLTLSKADYEKHKVYACEVTHQGLSSPVTKSFNRGEC

SEQ ID NO: 104 - DNA, 642 bp, Artificial Sequence
  source: /note="Description of Artificial Sequence: Synthetic polynucleotide"
gagatcgtgctgacccagagccccgccaccctgagcctgagccccggcgagagggccaccctgagctgcagggccagccagagcgtgcacagcagctacctggcctggtaccagcagaagcccggccaggcccccaggctgctgatctacggcgccagcagcagggccaccggcatccccgacaggttcagcggcagcggcagcggcaccgacttcaccctgaccatcagcaggctggagcccgaggacttcgccgtgtactactgccagcaggactacaggacccccagcttcggccagggcaccaggctggagatcaccaggaccgtggccgcccccagcgtgttcatcttcccccccagcgacgagcagctgaagagcggcaccgccagcgtggtgtgcctgctgaacaacttctaccccagggaggccaaggtgcagtggaaggtggacaacgccctgcagagcggcaacagccaggagagcgtgaccgagcaggacagcaaggacagcacctacagcctgagcagcaccctgaccctgagcaaggccgactacgagaagcacaaggtgtacgcctgcgaggtgacccaccagggcctgagcagccccgtgaccaagagcttcaacaggggcgagtgc

SEQ ID NO: 105 - protein, 107 aa, Artificial Sequence
  source: /note="Description of Artificial Sequence: Synthetic polypeptide"
EIVLTQSPATLSLSPGERATLSCRASQSVHSSYLAWYQQKPGQAPRLLIYGASSRATGIPDRFSGSGSGTDFTLTISRLEPEDFAVYYCQQDYRTPSFGQGTRLEIT

SEQ ID NO: 106 - DNA, 321 bp, Artificial Sequence
  source: /note="Description of Artificial Sequence: Synthetic polynucleotide"
gagatcgtgctgacccagagccccgccaccctgagcctgagccccggcgagagggccaccctgagctgcagggccagccagagcgtgcacagcagctacctggcctggtaccagcagaagcccggccaggcccccaggctgctgatctacggcgccagcagcagggccaccggcatccccgacaggttcagcggcagcggcagcggcaccgacttcaccctgaccatcagcaggctggagcccgaggacttcgccgtgtactactgccagcaggactacaggacccccagcttcggccagggcaccaggctggagatcacc

SEQ ID NO: 107 - protein, 5 aa, Artificial Sequence
  source: /note="Description of Artificial Sequence: Synthetic peptide"
WYEMY

SEQ ID NO: 108 - protein, 17 aa, Artificial Sequence
  source: /note="Description of Artificial Sequence: Synthetic peptide"
SISPSGGWTMYADSVKG

SEQ ID NO: 109 - protein, 13 aa, Artificial Sequence
  source: /note="Description of Artificial Sequence: Synthetic peptide"
PLYSSDGLSAGDI

SEQ ID NO: 110 - protein, 12 aa, Artificial Sequence
  source: /note="Description of Artificial Sequence: Synthetic peptide"
RASQSVHSSYLA

SEQ ID NO: 111 - protein, 7 aa, Artificial Sequence
  source: /note="Description of Artificial Sequence: Synthetic peptide"
GASSRAT

SEQ ID NO: 112 - protein, 8 aa, Artificial Sequence
  source: /note="Description of Artificial Sequence: Synthetic peptide"
QQDYRTPS

SEQ ID NO: 113 - protein, 12 aa, Artificial Sequence
  source: /note="Description of Artificial Sequence: Synthetic peptide"
RASQSVSSSYLA

SEQ ID NO: 114 - protein, 12 aa, Artificial Sequence
  source: /note="Description of Artificial Sequence: Synthetic peptide"
RASQSVHSSYLA

SEQ ID NO: 115 - protein, 8 aa, Artificial Sequence
  source: /note="Description of Artificial Sequence: Synthetic peptide"
QQSYSTPS

SEQ ID NO: 116 - protein, 8 aa, Artificial Sequence
  source: /note="Description of Artificial Sequence: Synthetic peptide"
QQSYRTPS

SEQ ID NO: 117 - protein, 8 aa, Artificial Sequence
  source: /note="Description of Artificial Sequence: Synthetic peptide"
QQDYSTPS

SEQ ID NO: 118 - protein, 8 aa, Artificial Sequence
  source: /note="Description of Artificial Sequence: Synthetic peptide"
QQDYRTPS